European Patent Application EP 4 566 627 A1, published June 11, 2025. Title: ニューロトリミンの機能阻害剤. Applicant: 国立大学法人　東京大学. Application JP. The sequence listing filed with the application follows.

SEQUENCE LISTING (35 sequences)

SEQ ID NO: 1 - DNA, 972 bp, Homo sapiens
  source 1..972: mol_type = other DNA
agcggagatgccaccttccccaaagctatggacaacgtgacggtccggcagggggagagcgccaccctcaggtgcactattgacaaccgggtcacccgggtggcctggctaaaccgcagcaccatcctctatgctgggaatgacaagtggtgcctggatcctcgcgtggtccttctgagcaacacccaaacgcagtacagcatcgagatccagaacgtggatgtgtatgacgagggcccttacacctgctcggtgcagacagacaaccacccaaagacctctagggtccacctcattgtgcaagtatctcccaaaattgtagagatttcttcagatatctccattaatgaagggaacaatattagcctcacctgcatagcaactggtagaccagagcctacggttacttggagacacatctctcccaaagcggttggctttgtgagtgaagacgaatacttggaaattcagggcatcaccagggagcagtcaggggactacgagtgcagtgcctccaatgacgtggccgcgcccgtggtacggagagtaaaggtcaccgtgaactatccaccatacatttcagaagccaagggtacaggtgtccccgtgggacaaaaggggacactgcagtgtgaagcctcagcagtcccctcagcagaattccagtggtacaaggatgacaaaagactgattgaaggaaagaaaggggtgaaagtggaaaacagacctttcctctcaaaactcatcttcttcaatgtctctgaacatgactatgggaactacacttgcgtggcctccaacaagctgggccacaccaatgccagcatcatgctatttgaagtgaaaactacagccctgaccccttggaaaggtccaggcgccgtcagcgaggtgagcaacggcacgtcgaggagggcaggctgcgtctggctgctgcctcttctggtcttgcacctgcttctcaaattttga

SEQ ID NO: 2 - protein, 323 aa, Homo sapiens
SGDATFPKAMDNVTVRQGESATLRCTIDNRVTRVAWLNRSTILYAGNDKWCLDPRVVLLSNTQTQYSIEIQNVDVYDEGPYTCSVQTDNHPKTSRVHLIVQVSPKIVEISSDISINEGNNISLTCIATGRPEPTVTWRHISPKAVGFVSEDEYLEIQGITREQSGDYECSASNDVAAPVVRRVKVTVNYPPYISEAKGTGVPVGQKGTLQCEASAVPSAEFQWYKDDKRLIEGKKGVKVENRPFLSKLIFFNVSEHDYGNYTCVASNKLGHTNASIMLFEVKTTALTPWKGPGAVSEVSNGTSRRAGCVWLLPLLVLHLLLKF

SEQ ID NO: 3 - protein, 8 aa, Homo sapiens
GYSFTSYW

SEQ ID NO: 4 - protein, 9 aa, Homo sapiens
IYPGDSDTR

SEQ ID NO: 5 - protein, 17 aa, Homo sapiens
ARQRFGEFAYYYYGLDV

SEQ ID NO: 6 - protein, 9 aa, Homo sapiens
TGAVTTSNY

SEQ ID NO: 7 - skipped

SEQ ID NO: 8 - protein, 9 aa, Homo sapiens
ALWYSTHYV

SEQ ID NO: 9 - protein, 8 aa, Homo sapiens
GYTLTELS

SEQ ID NO: 10 - protein, 9 aa, Homo sapiens
FDPEDGETI

SEQ ID NO: 11 - protein, 12 aa, Homo sapiens
ATYSSGWYALDY

SEQ ID NO: 12 - protein, 6 aa, Homo sapiens
QSVSIY

SEQ ID NO: 13 - skipped

SEQ ID NO: 14 - protein, 9 aa, Homo sapiens
QQRIKWPFT

SEQ ID NO: 15 - protein, 8 aa, Homo sapiens
GFTFSDYY

SEQ ID NO: 16 - protein, 9 aa, Homo sapiens
ISNDGSTIY

SEQ ID NO: 17 - protein, 24 aa, Homo sapiens
ARDYYGSGSFYPKPHYYYYYGMDV

SEQ ID NO: 18 - protein, 12 aa, Homo sapiens
QSVLYSSNNKNY

SEQ ID NO: 19 - skipped

SEQ ID NO: 20 - protein, 9 aa, Homo sapiens
QQYYSPPFT

SEQ ID NO: 21 - protein, 10 aa, Homo sapiens
GFSLSTSGVG

SEQ ID NO: 22 - protein, 8 aa, Homo sapiens
IYWDDDKR

SEQ ID NO: 23 - protein, 19 aa, Homo sapiens
AHSAYYDILTGYALDAFDI

SEQ ID NO: 24 - protein, 6 aa, Homo sapiens
QSVSSY

SEQ ID NO: 25 - skipped

SEQ ID NO: 26 - protein, 9 aa, Homo sapiens
RQRSNWPWT

SEQ ID NO: 27 - protein, 10 aa, Homo sapiens
GFSLSTSGVG

SEQ ID NO: 28 - protein, 8 aa, Homo sapiens
IYWDDDKR

SEQ ID NO: 29 - protein, 19 aa, Homo sapiens
AHSAYYDILTGYALDAFDI

SEQ ID NO: 30 - protein, 12 aa, Homo sapiens
QSVLYSSNNKIY

SEQ ID NO: 31 - skipped

SEQ ID NO: 32 - protein, 9 aa, Homo sapiens
QQYYSPPFT

SEQ ID NO: 33 - DNA, 21 bp, Mus musculus
  source 1..21: mol_type = genomic DNA
ctgaactgctacggggaagag

SEQ ID NO: 34 - DNA, 20 bp, Mus musculus
  source 1..20: mol_type = genomic DNA
gcagcgcatcgccttctatc

SEQ ID NO: 35 - DNA, 21 bp, Mus musculus
  source 1..21: mol_type = genomic DNA
ctcgggaaaaggcagtagcag